European Patent Specification EP 3 555 309 B1, published September 13, 2023. Title: EPIGENETIC MARKERS AND RELATED METHODS AND MEANS FOR THE DETECTION AND MANAGEMENT OF OVARIAN CANCER. Applicant: GATC Biotech AG Genedata AG UCL Business PLC. The sequence listing filed with the application follows.

SEQUENCE LISTING (159 sequences)

SEQ ID NO: 1 - DNA, 136 bp, Homo sapiens
catccggaggcccaggggtgaggacttcgccacgggaaggaggcacacgattcagcccatgacaccgccacctcggcgtggtgctgtagggggaagctcaggcactcaccgaggacaggacccggggaatccgctg

SEQ ID NO: 2 - DNA, 154 bp, Homo sapiens
gatattcggtggagagccgcagctgcccgccgcggggccccaggcgcagcacgctctcgcgcgtgggccgcagctggcagcacaggaagtccaggtggaagagcggcggcgtgggcggcccggcgcggcgcggcgagtgcgggctggtatcggc

SEQ ID NO: 3 - DNA, 111 bp, Homo sapiens
gttctatgggcgagctgctgcagtgcggctgccaggcgccccgcgggcgggcccctccccggccctccggcctgcccggcacccccggaccccctggccccgcgggctccc

SEQ ID NO: 4 - DNA, 140 bp, Homo sapiens
cccaggcctgacgtgggtcccccagggcggcgtcgccaaggcttagacgctttcgtgcaggagggacgacgactcccctcacgccttcgtggccccaactcggcgctctgctatctctgatccggtgaacacacctcaga

SEQ ID NO: 5 - DNA, 120 bp, Homo sapiens
gcgaagcaggagtagctgccgggccccacgagcctccgtccgttctggttcgggtttctccgagttttgctaccagccgaggctgtgcgggcaactgggtcagcctcccgtcaggagaga

SEQ ID NO: 6 - DNA, 120 bp, Homo sapiens
aactctgctgagtgagctcacaaacagggcataaccgagacgcgggaatgcctgggtcgccgcgcagtcaccgggcagggccgccctcccctgtgggtcagcaaaaacggtgtcaagtga

SEQ ID NO: 7 - DNA, 130 bp, Homo sapiens
actccgccacacacacagctgtacccggcacaacacgcggccacaggtcacctcaggtcgcctcgggtgctcctcccgcagccccacgtagacagaagacattcctcgggcctgggtgcccagcctcccg

SEQ ID NO: 8 - DNA, 120 bp, Homo sapiens
gaggtaatggaagcggccatccttgtcctcgctccgcgcctggctgaagcgatcggggtcgaacacgttcacgtctttgaacacgggcgctgtgtcatgggtgtcccggatgctatacat

SEQ ID NO: 9 - DNA, 137 bp, Homo sapiens
gcgggcacctgtagtcccagctactcgggaggctgaggcgggagaatggcgtgaacccgggaggcggagcttgcagcgagccgagatcgcgccaccgcactccagcctgggcgacagagcgagactccgtctaaaaa

SEQ ID NO: 10 - DNA, 137 bp, Homo sapiens
tccccggagtccggagctcaggccagtggcagtcgacccagcccccgagactccctcacgccgctccaaaaccaaaacggagcccaacacgaagctgggtgaagccgtagcttgcaggagccagggagatgcgctct

SEQ ID NO: 11 - DNA, 136 bp, Homo sapiens
gactctgtctcaaaaaagaaaaaaatagggccgggcgcggtggctcacgcctgtcatcccagcactttgggaggccgaggcgggtggatcacgaggtcgggagatcgataccatcctgggtaacacggtgaaaccc

SEQ ID NO: 12 - DNA, 138 bp, Homo sapiens
gactcgcgaggttttccagcagctcattccgggacggcggtgtctagtccagtccagggtaactgggctctctgagagtccgacctccatcggtctgggagcgagtggttcgagttcagatgctgggaaccgtcgctt

SEQ ID NO: 13 - DNA, 138 bp, Homo sapiens
taacccatttctttattaaattgcatgaagaaggccgggcgcggtggctcacgcctgtaatcccagcactttgggaggccgaggcgggcggatcacgaggtcaggagatcgagaccacggtgaaaccccgtctctact

SEQ ID NO: 14 - DNA, 142 bp, Homo sapiens
ggcaggagcgccccactatgcgcaagcccgtggcctggagagcgctgaaggtgggagggggaagaggggcagaacccccgcgggagcgagcgcacagctgccgccccgtggccgcttcgggaatcgctggctccggctctgg

SEQ ID NO: 15 - DNA, 135 bp, Homo sapiens
ctgcagaagcgcactttgctgaacaccccgaggacgtgcctctcgcacagggagcgcccgtctttgctggggctggagcggcgcttggaggccgacactcggtcgctgttggactccctcgcctgccgcttctgc

SEQ ID NO: 16 - DNA, 146 bp, Homo sapiens
cgtgttagccaggatggtctcgacctcctgacctcgtgatcagcccgcctcggcctcccaaagtgctgggattaaaggcgtgagccaccgcgccgggccgagactctgtcttaaaaaaaaaaggcctgggctgtggcactttggga

SEQ ID NO: 17 - DNA, 141 bp, Homo sapiens
agagttgcactccgaagactccagattccgagagttgcggaaacgctacgaggacctgctaaccaggctgcgggccaaccagagctgggaagattcgaacaccgacctcgtcccggcccctgcagtccggatactcacgcc

SEQ ID NO: 18 - DNA, 109 bp, Homo sapiens
gtcagacgagagcctggggtcaatgtcgaggtggagcgacgctggcacggcaaccctgagcctgcgcggcccggcgctatcccctggctctccgctgctggctggaccc

SEQ ID NO: 19 - DNA, 144 bp, Homo sapiens
cggtaggtcatccagcagcagggctccacgtcggtctcgtcgatgccccagaaggccagctcctcctcgaagagcggcccgcacacgtctgcggggcagtgcagcttgccggtgcggtagtaattgagcacataggcgaagacg

SEQ ID NO: 20 - DNA, 115 bp, Homo sapiens
aatcagcccagcaaccggcgaccccaagcgcggcgaccgcaaagggagtgcttgcccatccgcgtttgaaagcagactttttctcggcaggaacacaggactcacctgccagtgg

SEQ ID NO: 21 - DNA, 148 bp, Homo sapiens
gtgcgaacaagaccgggcgtttcgccgccgacgcgaaggggctgtctgtgcgcggcgttgcgggccctccgcgcgtggggtgtgcgtgtgcgtgttcgggttcggttctgtgtgtgcaccgcgggcctgctcagagtcgggaccaccg

SEQ ID NO: 22 - DNA, 121 bp, Homo sapiens
atattaatcttgtccgggcacggtggctcacgcctgtaatcccagcactttgggaggccgaggcgggcggatcacgaggtcaggagatcgagaccatcctggcgaacatggtgaaacctcg

SEQ ID NO: 23 - DNA, 92 bp, Homo sapiens
tgcatacagattactgtaggaccatttcctgtgccttttaaaatttccttttctcgttttatttcacatattcctttgttttttacaactcc

SEQ ID NO: 24 - DNA, 103 bp, Homo sapiens
ccgctcgggaatgggaatatagctacatatgggaaaacgcggtgcagggagaaaaccaattcagtgaggagcggaggcgcaggactgtggagtgtgcatccgg

SEQ ID NO: 25 - DNA, 94 bp, Homo sapiens
ctgcttaaaggcgcagaggagcagctgggaacgagaacaaagcggccaggcccccctcggaggaaggaaggagagagccccaggaaacagctga

SEQ ID NO: 26 - DNA, 101 bp, Homo sapiens
ggatgaaggattcctgcatcactgtgatggccatggcgctgctgtctgggttctttttcttcggtaggcaagggaggaggcaggggaagggacatgtgtct

SEQ ID NO: 27 - DNA, 70 bp, Homo sapiens
taggctacaggaagaggcatttcctatagatgacggctgtaaaattttaagctgagttcctccaggaagt

SEQ ID NO: 28 - DNA, 84 bp, Homo sapiens
aagagagagtggttgataatcagtagagagaggtttctaactcacggaagtgtttgcaatacaacctctttgtacatcagctgt

SEQ ID NO: 29 - DNA, 97 bp, Homo sapiens
ggtccccctccccgagccatgaagagctgcctgcggccatcttggccctcgcaccccgtctctgtcaccccaggcccctgtaacttgcttaacgctt

SEQ ID NO: 30 - DNA, 86 bp, Homo sapiens
gaagcttgacactcctggccccaaacactgcctggctacaacacgatatccagggacagataccttccatgtacagcaagctgtgg

SEQ ID NO: 31 - DNA, 91 bp, Homo sapiens
ggggggactgtcgttaattcactgcctaatgaccgcggcccgcgcgctccgagtaatcgggtgatgtatgtggactgtgcacacctcgtgg

SEQ ID NO: 32 - DNA, 136 bp, Artificial Sequence
  DMR 141
tattyggaggtttaggggtgaggatttygttaygggaaggaggtataygatttagtttatgatatygttatttyggygtggtgttgtagggggaagtttaggtatttatygaggataggattyggggaattygttg

SEQ ID NO: 33 - DNA, 154 bp, Artificial Sequence
  DMR 204
gatattyggtggagagtygtagttgttygtygyggggttttaggygtagtaygttttygygygtgggtygtagttggtagtataggaagtttaggtggaagagyggyggygtgggyggttyggygyggygyggygagtgygggttggtatyggt

SEQ ID NO: 34 - DNA, 111 bp, Artificial Sequence
  DMR 228
gttttatgggygagttgttgtagtgyggttgttaggygtttygygggygggttttttttyggtttttyggtttgttyggtattttyggattttttggtttygygggttttt

SEQ ID NO: 35 - DNA, 140 bp, Artificial Sequence
  DMR 144
tttaggtttgaygtgggttttttagggyggygtygttaaggtttagaygttttygtgtaggagggaygaygattttttttaygttttygtggttttaattyggygttttgttatttttgattyggtgaatatattttaga

SEQ ID NO: 36 - DNA, 120 bp, Artificial Sequence
  DMR 123
gygaagtaggagtagttgtygggttttaygagttttygttygttttggttygggttttttygagttttgttattagtygaggttgtgygggtaattgggttagtttttygttaggagaga

SEQ ID NO: 37 - DNA, 120 bp, Artificial Sequence
  DMR 129
aattttgttgagtgagtttataaatagggtataatygagaygygggaatgtttgggtygtygygtagttatygggtagggtygtttttttttgtgggttagtaaaaayggtgttaagtga

SEQ ID NO: 38 - DNA, 130 bp, Artificial Sequence
  DMR 137
atttygttatatatatagttgtattyggtataataygyggttataggttattttaggtygtttygggtgtttttttygtagttttaygtagatagaagatatttttygggtttgggtgtttagtttttyg

SEQ ID NO: 39 - DNA, 120 bp, Artificial Sequence
  DMR 148
gaggtaatggaagyggttatttttgttttygtttygygtttggttgaagygatyggggtygaataygtttaygtttttgaataygggygttgtgttatgggtgtttyggatgttatatat

SEQ ID NO: 40 - DNA, 137 bp, Artificial Sequence
  DMR 150
gygggtatttgtagttttagttattygggaggttgaggygggagaatggygtgaattygggaggyggagtttgtagygagtygagatygygttatygtattttagtttgggygatagagygagatttygtttaaaaa

SEQ ID NO: 41 - DNA, 137 bp, Artificial Sequence
  DMR 154
ttttyggagttyggagtttaggttagtggtagtygatttagttttygagatttttttaygtygttttaaaattaaaayggagtttaataygaagttgggtgaagtygtagtttgtaggagttagggagatgygtttt

SEQ ID NO: 42 - DNA, 136 bp, Artificial Sequence
  DMR 158
gattttgttttaaaaaagaaaaaaatagggtygggygyggtggtttaygtttgttattttagtattttgggaggtygaggygggtggattaygaggtygggagatygatattattttgggtaatayggtgaaattt

SEQ ID NO: 43 - DNA, 138 bp, Artificial Sequence
  DMR 164
gattygygaggttttttagtagtttatttygggayggyggtgtttagtttagtttagggtaattgggttttttgagagttygatttttatyggtttgggagygagtggttygagtttagatgttgggaatygtygttt

SEQ ID NO: 44 - DNA, 138 bp, Artificial Sequence
  DMR 176
taatttatttttttattaaattgtatgaagaaggtygggygyggtggtttaygtttgtaattttagtattttgggaggtygaggygggyggattaygaggttaggagatygagattayggtgaaatttygtttttatt

SEQ ID NO: 45 - DNA, 142 bp, Artificial Sequence
  DMR 178
ggtaggagygttttattatgygtaagttygtggtttggagagygttgaaggtgggagggggaagaggggtagaattttygygggagygagygtatagttgtygtttygtggtygtttygggaatygttggtttyggttttgg

SEQ ID NO: 46 - DNA, 135 bp, Artificial Sequence
  DMR 180
ttgtagaagygtattttgttgaatatttygaggaygtgtttttygtatagggagygttygtttttgttggggttggagyggygtttggaggtygatattyggtygttgttggattttttygtttgtygtttttgt

SEQ ID NO: 47 - DNA, 146 bp, Artificial Sequence
  DMR 186
ygtgttagttaggatggtttygattttttgatttygtgattagttygtttyggttttttaaagtgttgggattaaaggygtgagttatygygtygggtygagattttgttttaaaaaaaaaaggtttgggttgtggtattttggga

SEQ ID NO: 48 - DNA, 141 bp, Artificial Sequence
  DMR 188
agagttgtatttygaagattttagatttygagagttgyggaaaygttaygaggatttgttaattaggttgygggttaattagagttgggaagattygaatatygatttygtttyggtttttgtagttyggatatttaygtt

SEQ ID NO: 49 - DNA, 109 bp, Artificial Sequence
  DMR 190
gttagaygagagtttggggttaatgtygaggtggagygaygttggtayggtaattttgagtttgygyggttyggygttattttttggtttttygttgttggttggattt

SEQ ID NO: 50 - DNA, 144 bp, Artificial Sequence
  DMR 192
yggtaggttatttagtagtagggttttaygtyggtttygtygatgttttagaaggttagttttttttygaagagyggttygtataygtttgyggggtagtgtagtttgtyggtgyggtagtaattgagtatataggygaagayg

SEQ ID NO: 51 - DNA, 115 bp, Artificial Sequence
  DMR 200
aattagtttagtaatyggygattttaagygyggygatygtaaagggagtgtttgtttattygygtttgaaagtagattttttttyggtaggaatataggatttatttgttagtgg

SEQ ID NO: 52 - DNA, 148 bp, Artificial Sequence
  DMR 202
gtgygaataagatygggygtttygtygtygaygygaaggggttgtttgtgygyggygttgygggtttttygygygtggggtgtgygtgtgygtgttygggttyggttttgtgtgtgtatygygggtttgtttagagtygggattatyg

SEQ ID NO: 53 - DNA, 121 bp, Artificial Sequence
  DMR 208
atattaattttgttygggtayggtggtttaygtttgtaattttagtattttgggaggtygaggygggyggattaygaggttaggagatygagattattttggygaatatggtgaaatttyg

SEQ ID NO: 54 - DNA, 92 bp, Artificial Sequence
  DMR 210
tgtatatagattattgtaggattattttttgtgttttttaaaatttttttttttygttttattttatatatttttttgttttttataatttt

SEQ ID NO: 55 - DNA, 103 bp, Artificial Sequence
  DMR 213
tygttygggaatgggaatatagttatatatgggaaaaygyggtgtagggagaaaattaatttagtgaggagyggaggygtaggattgtggagtgtgtattygg

SEQ ID NO: 56 - DNA, 94 bp, Artificial Sequence
  DMR 214
ttgtttaaaggygtagaggagtagttgggaaygagaataaagyggttaggtttttttyggaggaaggaaggagagagttttaggaaatagttga

SEQ ID NO: 57 - DNA, 101 bp, Artificial Sequence
  DMR 219
ggatgaaggatttttgtattattgtgatggttatggygttgttgtttgggtttttttttttyggtaggtaagggaggaggtaggggaagggatatgtgttt

SEQ ID NO: 58 - DNA, 70 bp, Artificial Sequence
  DMR 222
taggttataggaagaggtattttttatagatgayggttgtaaaattttaagttgagtttttttaggaagt

SEQ ID NO: 59 - DNA, 84 bp, Artificial Sequence
  DMR 223
aagagagagtggttgataattagtagagagaggtttttaatttayggaagtgtttgtaatataatttttttgtatattagttgt

SEQ ID NO: 60 - DNA, 97 bp, Artificial Sequence
  DMR 224
ggttttttttttygagttatgaagagttgtttgyggttattttggttttygtatttygtttttgttattttaggtttttgtaatttgtttaaygttt

SEQ ID NO: 61 - DNA, 86 bp, Artificial Sequence
  DMR 225
gaagtttgatatttttggttttaaatattgtttggttataataygatatttagggatagatattttttatgtatagtaagttgtgg

SEQ ID NO: 62 - DNA, 91 bp, Artificial Sequence
  DMR 226
ggggggattgtygttaatttattgtttaatgatygyggttygygygtttygagtaatygggtgatgtatgtggattgtgtatatttygtgg

SEQ ID NO: 63 - DNA, 84 bp, Artificial Sequence
  DMR 141
cgttacgggaaggaggtatacgatttagtttatgatatcgttatttcggcgtggtgttgtagggggaagtttaggtatttatcg

SEQ ID NO: 64 - DNA, 107 bp, Artificial Sequence
  DMR 204
cgtcgcggggttttaggcgtagtacgttttcgcgcgtgggtcgtagttggtagtataggaagtttaggtggaagagcggcggcgtgggcggttcggcgcggygyggt

SEQ ID NO: 65 - DNA, 62 bp, Artificial Sequence
  DMR 228
yggttgttaggcgtttcgcgggygggttttttttcggtttttcggtttgttcggtattttcg

SEQ ID NO: 66 - DNA, 80 bp, Artificial Sequence
  DMR 144
ggcggcgtcgttaaggtttagacgttttcgtgtaggagggacgacgattttttttacgttttcgtggttttaattcggcg

SEQ ID NO: 67 - DNA, 61 bp, Artificial Sequence
  DMR 123
tgagtttttgtttgttttggtttgggtttttttgagttttgttattagttgaggttgtgtg

SEQ ID NO: 68 - DNA, 61 bp, Artificial Sequence
  DMR 129
tygagatgtgggaatgtttgggtygtygtgtagttattgggtagggtygtttttttttgtg

SEQ ID NO: 69 - DNA, 73 bp, Artificial Sequence
  DMR 137
tgtggttataggttattttaggttgttttgggtgttttttttgtagttttatgtagatagaagatattttttg

SEQ ID NO: 70 - DNA, 64 bp, Artificial Sequence
  DMR 148
ttttygttttgtgtttggttgaagtgattggggtygaataygtttaygtttttgaatatgggyg

SEQ ID NO: 71 - DNA, 88 bp, Artificial Sequence
  DMR 150
tgggaggttgaggtgggagaatggtgtgaatttgggaggtggagtttgtagtgagttgagattgtgttattgtattttagtttgggtg

SEQ ID NO: 72 - DNA, 76 bp, Artificial Sequence
  DMR 154
gtygatttagttttcgagatttttttacgtcgttttaaaattaaaacggagtttaatacgaagttgggtgaagtcg

SEQ ID NO: 73 - DNA, 76 bp, Artificial Sequence
  DMR 158
ygggygtggtggtttatgtttgttattttagtattttgggaggttgaggtgggtggattatgaggttgggagattg

SEQ ID NO: 74 - DNA, 83 bp, Artificial Sequence
  DMR 164
ygggayggyggtgtttagtttagtttagggtaattgggttttttgagagttcgatttttatcggtttgggagcgagtggttcg

SEQ ID NO: 75 - DNA, 76 bp, Artificial Sequence
  DMR 176
ygggtgtggtggtttaygtttgtaattttagtattttgggaggttgaggtgggyggattaygaggttaggagatyg

SEQ ID NO: 76 - DNA, 91 bp, Artificial Sequence
  DMR 178
ygtggtttggagagygttgaaggtgggagggggaagaggggtagaattttygcgggagcgagcgtatagttgtcgtttygtggtcgtttyg

SEQ ID NO: 77 - DNA, 71 bp, Artificial Sequence
  DMR 180
ygtgtttttygtatagggagcgttygtttttgttggggttggagcggcgtttggaggtcgatattcggtcg

SEQ ID NO: 78 - DNA, 88 bp, Artificial Sequence
  DMR 186
ygtgattagttygttttggttttttaaagtgttgggattaaaggtgtgagttattgtgttgggttgagattttgttttaaaaaaaaaa

SEQ ID NO: 79 - DNA, 87 bp, Artificial Sequence
  DMR 188
tgagagttgyggaaaygttaygaggatttgttaattaggttgygggttaattagagttgggaagatttgaatattgattttgtttyg

SEQ ID NO: 80 - DNA, 56 bp, Artificial Sequence
  DMR 190
cgaggtggagcgacgttggtacggtaattttgagtttgcgcggttcggcgttattt

SEQ ID NO: 81 - DNA, 88 bp, Artificial Sequence
  DMR 192
cgtcggtttcgtcgatgttttagaaggttagttttttttcgaagagcggttcgtatacgtttgcggggtagtgtagtttgtcggtgcg

SEQ ID NO: 82 - DNA, 58 bp, Artificial Sequence
  DMR 200
cgcggcgatcgtaaagggagtgtttgtttattcgcgtttgaaagtagattttttttcg

SEQ ID NO: 83 - DNA, 101 bp, Artificial Sequence
  DMR 202
ygtygtygaygygaaggggttgtttgtgcgcggygttgygggtttttcgcgcgtggggtgtgcgtgtgcgtgttcgggttcggttttgtgtgtgtatcgcg

SEQ ID NO: 84 - DNA, 61 bp, Artificial Sequence
  DMR 208
atgtttgtaattttagtattttgggaggttgaggtgggtggattatgaggttaggagattg

SEQ ID NO: 85 - DNA, 30 bp, Artificial Sequence
  DMR 210
tttttaaaatttttttttttcgttttattt

SEQ ID NO: 86 - DNA, 49 bp, Artificial Sequence
  DMR 213
gaaaacgcggtgtagggagaaaattaatttagtgaggagcggaggcgta

SEQ ID NO: 87 - DNA, 34 bp, Artificial Sequence
  DMR 214
gaacgagaataaagcggttaggtttttttcggag

SEQ ID NO: 88 - DNA, 41 bp, Artificial Sequence
  DMR 219
gcgttgttgtttgggtttttttttttcggtaggtaagggag

SEQ ID NO: 89 - DNA, 10 bp, Artificial Sequence
  DMR 222
  misc_feature 1..2: /note="n can be any nucleotide"
  misc_feature 9..10: /note="n can be any nucleotide"
nnacggttnn

SEQ ID NO: 90 - DNA, 23 bp, Artificial Sequence
  DMR 223
agagaggtttttaatttacggaa

SEQ ID NO: 91 - DNA, 34 bp, Artificial Sequence
  DMR 224
tttgcggttattttggttttcgtatttcgttttt

SEQ ID NO: 92 - DNA, 19 bp, Artificial Sequence
  DMR 225
gttataatacgatatttag

SEQ ID NO: 93 - DNA, 29 bp, Artificial Sequence
  DMR 226
attgtggtttgtgtgttttgagtaattgg

SEQ ID NO: 94 - DNA, 27 bp, Artificial Sequence
  DMR 141 for
tattyggaggtttaggggtgaggattt

SEQ ID NO: 95 - DNA, 27 bp, Artificial Sequence
  DMR 204 for
gatattyggtggagagtygtagttgtt

SEQ ID NO: 96 - DNA, 25 bp, Artificial Sequence
  DMR 228 for
gttttatgggygagttgttgtagtg

SEQ ID NO: 97 - DNA, 25 bp, Artificial Sequence
  DMR 144 for
tttaggtttgaygtgggttttttag

SEQ ID NO: 98 - DNA, 28 bp, Artificial Sequence
  DMR 123 for
gygaagtaggagtagttgtygggtttta

SEQ ID NO: 99 - DNA, 34 bp, Artificial Sequence
  DMR 129 for
aattttgttgagtgagtttataaatagggtataa

SEQ ID NO: 100 - DNA, 35 bp, Artificial Sequence
  DMR 137 for
atttygttatatatatagttgtattyggtataata

SEQ ID NO: 101 - DNA, 25 bp, Artificial Sequence
  DMR 148 for
gaggtaatggaagyggttatttttg

SEQ ID NO: 102 - DNA, 25 bp, Artificial Sequence
  DMR 150 for
gygggtatttgtagttttagttatt

SEQ ID NO: 103 - DNA, 31 bp, Artificial Sequence
  DMR 154 for
ttttyggagttyggagtttaggttagtggta

SEQ ID NO: 104 - DNA, 31 bp, Artificial Sequence
  DMR 158 for
gattttgttttaaaaaagaaaaaaatagggt

SEQ ID NO: 105 - DNA, 29 bp, Artificial Sequence
  DMR 164 for
gattygygaggttttttagtagtttattt

SEQ ID NO: 106 - DNA, 35 bp, Artificial Sequence
  DMR 176 for
taatttatttttttattaaattgtatgaagaaggt

SEQ ID NO: 107 - DNA, 28 bp, Artificial Sequence
  DMR 178 for
ggtaggagygttttattatgygtaagtt

SEQ ID NO: 108 - DNA, 34 bp, Artificial Sequence
  DMR 180 for
ttgtagaagygtattttgttgaatatttygagga

SEQ ID NO: 109 - DNA, 34 bp, Artificial Sequence
  DMR 186 for
ygtgttagttaggatggtttygattttttgattt

SEQ ID NO: 110 - DNA, 28 bp, Artificial Sequence
  DMR 188 for
agagttgtatttygaagattttagattt

SEQ ID NO: 111 - DNA, 26 bp, Artificial Sequence
  DMR 190 for
gttagaygagagtttggggttaatgt

SEQ ID NO: 112 - DNA, 28 bp, Artificial Sequence
  DMR 192 for
yggtaggttatttagtagtagggtttta

SEQ ID NO: 113 - DNA, 28 bp, Artificial Sequence
  DMR 200 for
aattagtttagtaatyggygattttaag

SEQ ID NO: 114 - DNA, 22 bp, Artificial Sequence
  DMR 202 for
gtgygaataagatygggygttt

SEQ ID NO: 115 - DNA, 29 bp, Artificial Sequence
  DMR 208 for
atattaattttgttygggtayggtggttt

SEQ ID NO: 116 - DNA, 28 bp, Artificial Sequence
  DMR 210 for
ggagttgtaaaaaataaaggaatatgtg

SEQ ID NO: 117 - DNA, 32 bp, Artificial Sequence
  DMR 213 for
tygttygggaatgggaatatagttatatatgg

SEQ ID NO: 118 - DNA, 28 bp, Artificial Sequence
  DMR 214 for
ttgtttaaaggygtagaggagtagttgg

SEQ ID NO: 119 - DNA, 35 bp, Artificial Sequence
  DMR 219 for
ggatgaaggatttttgtattattgtgatggttatg

SEQ ID NO: 120 - DNA, 32 bp, Artificial Sequence
  DMR 222 for
taggttataggaagaggtattttttatagatg

SEQ ID NO: 121 - DNA, 26 bp, Artificial Sequence
  DMR 223 for
aagagagagtggttgataattagtag

SEQ ID NO: 122 - DNA, 29 bp, Artificial Sequence
  DMR 224 for
ggttttttttttygagttatgaagagttg

SEQ ID NO: 123 - DNA, 34 bp, Artificial Sequence
  DMR 225 for
gaagtttgatatttttggttttaaatattgtttg

SEQ ID NO: 124 - DNA, 31 bp, Artificial Sequence
  DMR 226 for
ggggggattgtygttaatttattgtttaatg

SEQ ID NO: 125 - DNA, 25 bp, Artificial Sequence
  DMR 141 rev
caacraattccccraatcctatcct

SEQ ID NO: 126 - DNA, 20 bp, Artificial Sequence
  DMR 204 rev
accrataccaacccrcactc

SEQ ID NO: 127 - DNA, 24 bp, Artificial Sequence
  DMR 228 rev
aaaaacccrcraaaccaaaaaatc

SEQ ID NO: 128 - DNA, 35 bp, Artificial Sequence
  DMR 144 rev
tctaaaatatattcaccraatcaaaaataacaaaa

SEQ ID NO: 129 - DNA, 31 bp, Artificial Sequence
  DMR 123 rev
tctctcctaacraaaaactaacccaattacc

SEQ ID NO: 130 - DNA, 25 bp, Artificial Sequence
  DMR 129 rev
tcacttaacaccrtttttactaacc

SEQ ID NO: 131 - DNA, 22 bp, Artificial Sequence
  DMR 137 rev
craaaaactaaacacccaaacc

SEQ ID NO: 132 - DNA, 31 bp, Artificial Sequence
  DMR 148 rev
atatataacatccraaacacccataacacaa

SEQ ID NO: 133 - DNA, 24 bp, Artificial Sequence
  DMR 150 rev
tttttaaacraaatctcrctctat

SEQ ID NO: 134 - DNA, 30 bp, Artificial Sequence
  DMR 154 rev
aaaacrcatctccctaactcctacaaacta

SEQ ID NO: 135 - DNA, 29 bp, Artificial Sequence
  DMR 158 rev
aaatttcaccrtattacccaaaataatat

SEQ ID NO: 136 - DNA, 26 bp, Artificial Sequence
  DMR 164 rev
aaacracrattcccaacatctaaact

SEQ ID NO: 137 - DNA, 27 bp, Artificial Sequence
  DMR 176 rev
aataaaaacraaatttcaccrtaatct

SEQ ID NO: 138 - DNA, 23 bp, Artificial Sequence
  DMR 178 rev
ccaaaaccraaaccaacrattcc

SEQ ID NO: 139 - DNA, 30 bp, Artificial Sequence
  DMR 180 rev
acaaaaacracaaacraaaaaatccaacaa

SEQ ID NO: 140 - DNA, 24 bp, Artificial Sequence
  DMR 186 rev
tcccaaaataccacaacccaaacc

SEQ ID NO: 141 - DNA, 26 bp, Artificial Sequence
  DMR 188 rev
aacrtaaatatccraactacaaaaac

SEQ ID NO: 142 - DNA, 27 bp, Artificial Sequence
  DMR 190 rev
aaatccaaccaacaacraaaaaccaaa

SEQ ID NO: 143 - DNA, 28 bp, Artificial Sequence
  DMR 192 rev
crtcttcrcctatatactcaattactac

SEQ ID NO: 144 - DNA, 29 bp, Artificial Sequence
  DMR 200 rev
ccactaacaaataaatcctatattcctac

SEQ ID NO: 145 - DNA, 25 bp, Artificial Sequence
  DMR 202 rev
crataatcccractctaaacaaacc

SEQ ID NO: 146 - DNA, 31 bp, Artificial Sequence
  DMR 208 rev
craaatttcaccatattcrccaaaataatct

SEQ ID NO: 147 - DNA, 34 bp, Artificial Sequence
  DMR 210 rev
tacatacaaattactataaaaccatttcctatac

SEQ ID NO: 148 - DNA, 22 bp, Artificial Sequence
  DMR 213 rev
ccraatacacactccacaatcc

SEQ ID NO: 149 - DNA, 32 bp, Artificial Sequence
  DMR 214 rev
tcaactatttcctaaaactctctccttccttc

SEQ ID NO: 150 - DNA, 25 bp, Artificial Sequence
  DMR 219 rev
aaacacatatcccttcccctacctc

SEQ ID NO: 151 - DNA, 32 bp, Artificial Sequence
  DMR 222 rev
acttcctaaaaaaactcaacttaaaattttac

SEQ ID NO: 152 - DNA, 35 bp, Artificial Sequence
  DMR 223 rev
acaactaatatacaaaaaaattatattacaaacac

SEQ ID NO: 153 - DNA, 34 bp, Artificial Sequence
  DMR 224 rev
aaacrttaaacaaattacaaaaacctaaaataac

SEQ ID NO: 154 - DNA, 33 bp, Artificial Sequence
  DMR 225 rev
ccacaacttactatacataaaaaatatctatcc

SEQ ID NO: 155 - DNA, 31 bp, Artificial Sequence
  DMR 226 rev
ccacraaatatacacaatccacatacatcac

SEQ ID NO: 156 - DNA, 84 bp, Homo sapiens
cgccacgggaaggaggcacacgattcagcccatgacaccgccacctcggcgtggtgctgtagggggaagctcaggcactcaccg

SEQ ID NO: 157 - DNA, 107 bp, Homo sapiens
cgccgcggggccccaggcgcagcacgctctcgcgcgtgggccgcagctggcagcacaggaagtccaggtggaagagcggcggcgtgggcggcccggcgcggcgcggc

SEQ ID NO: 158 - DNA, 62 bp, Homo sapiens
cggctgccaggcgccccgcgggcgggcccctccccggccctccggcctgcccggcacccccg

SEQ ID NO: 159 - DNA, 80 bp, Homo sapiens
ggcggcgtcgccaaggcttagacgctttcgtgcaggagggacgacgactcccctcacgccttcgtggccccaactcggcg